European Patent Application EP 4 681 723 A1, published January 21, 2026. Title: 用于治疗三阴性乳癌的药物组合物. Applicant: 侯明宏. The sequence listing filed with the application follows.

SEQUENCE LISTING (3 sequences)

SEQ ID NO: 1 - DNA, 12 bp, synthetic construct
  source 1..12: mol_type = other DNA; organism (original language) = 人工合成
aaaagaagaaaa

SEQ ID NO: 2 - DNA, 12 bp, synthetic construct
  source 1..12: mol_type = other DNA
aaaagccgaaaa

SEQ ID NO: 3 - DNA, 12 bp, synthetic construct
  source 1..12: mol_type = other DNA
aaagcacgaaaa